European Patent Application EP 4 245 320 A2, published September 20, 2023. Title: METHODS AND COMPOSITIONS FOR IMMUNE PROTECTION AGAINST EXTRA-INTESTINAL PATHOGENIC E. COLI. Applicant: GLAXOSMITHKLINE BIOLOGICALS SA. Application EP, filed August 24, 2016. The sequence listing filed with the application follows.

SEQUENCE LISTING (3 sequences)

SEQ ID NO: 1 - protein, 652 aa, synthetic construct
GSGGGDQNATGSGGGKLAEEAFDLWNECAKACVLDLKDGVRSSRMSVDPAIADTNGQGVLHYSMVLEGGNDALKLAIDNALSITSDGLTIRLEGGVEPNKPVRYSYTRQARGSWSLNWLVPIGHEKPSNIKVFIHELNAGNQLSHMSPIYTIEMGDELLAKLARDATFFVRAHESNEMQPTLAISHAGVSVVMAQAQPRREKRWSEWASGKVLCLLDPLDGVYNYLAQQRCNLDDTWEGKIYRVLAGNPAKHDLDIKDNNNSTPTVISHRLHFPEGGSLAALTAHQACHLPLEAFTRHRQPRGWEQLEQCGYPVQRLVALYLAARLSWNQVDQVIRNALASPGSGGDLGEAIREQPEQARLALTLAAAESERFVRQGTGNDEAGAASADVVSLTCPVAKDQNRTKGECAGPADSGDALLERNYPTGAEFLGDGGDVSFSTRGTQNWTVERLLQAHRQLEERGYVFVGYHGTFLEAAQSIVFGGVRARSQDLDAIWRGFYIAGDPALAYGYAQDQEPDARGRIRNGALLRVYVPRWSLPGFYRTGLTLAAPEAAGEVERLIGHPLPLRLDAITGPEEEGGRVTILGWPLAERTVVIPSAIPTDPRNVGGDLDPSSIPDKEQAISALPDYASQPGKPPREDLKLGSGGGDQNAT

SEQ ID NO: 2-3 - skipped (2 entries)